European Patent Specification EP 3 598 980 B1, published January 28, 2026. Title: Compositions and Methods to Regulate Renalase in the Treatment of Diseases and Disorders. Applicant: Yale University Desir, Gary Hunt, Abigail O-Rear, Jessica Flynn, Peter. Application EP15812170.7. The sequence listing filed with the application follows.

SEQUENCE LISTING (95 sequences)

SEQ ID NO: 1 - protein, 17 aa, homo sapiens
AVWDKADDSGGRMTTAC

SEQ ID NO: 2 - protein, 17 aa, homo sapiens
AVWDKAEDSGGRMTTAC

SEQ ID NO: 3 - protein, 16 aa, homo sapiens
CTPHYAKKHQRFYDEL

SEQ ID NO: 4 - protein, 21 aa, homo sapiens
CIRFVSIDNKKRNIESSEIGP

SEQ ID NO: 5 - protein, 14 aa, homo sapiens
PGQMTLHHKPFLAC

SEQ ID NO: 6 - protein, 10 aa, homo sapiens
CVLEALKNYI

SEQ ID NO: 7 - protein, 9 aa, homo sapiens
PSAGVILGC

SEQ ID NO: 8 - protein, 342 aa, homo sapiens
MAQVLIVGAGMTGSLCAALLRRQTSGPLYLAVWDKAEDSGGRMTTACSPHNPQCTADLGAQYITCTPHYAKKHQRFYDELLAYGVLRPLSSPIEGMVMKEGDCNFVAPQGISSIIKHYLKESGAEVYFRHRVTQINLRDDKWEVSKQTGSPEQFDLIVLTMPVPEILQLQGDITTLISECQRQQLEAVSYSSRYALGLFYEAGTKIDVPWAGQYITSNPCIRFVSIDNKKRNIESSEIGPSLVIHTTVPFGVTYLEHSIEDVQELVFQQLENILPGLPQPIATKCQKWRHSQVTNAAANCPGQMTLHHKPFLACGGDGFTQSNFDGCITSALCVLEALKNYI

SEQ ID NO: 9 - protein, 459 aa, oryctolagus cuniculus
METGLRWLLLVAVLKGVQCQSVEESGGRLVTPGTPLTLTCTVSGFSLSSFAVGWVRQAPGKGLEYIGIISSVGITRYASWAAGRFTISKTSTTVDLKITSPTTEDTATYFCARYGYSGDVNRLDLWGQGTLVTVSSGQPKAPSVFPLAPCCGDTPSSTVTLGCLVKGYLPEPVTVTWNSGTLTNGVRTFPSVRQSSGLYSLSSVVSVTSSSQPVTCNVAHPATNTKVDKTVAPSTCSKPTCPPPELLGGPSVFIFPPKPKDTLMISRTPEVTCVVVDVSQDDPEVQFTWYINNEQVRTARPPLREQQFNSTIRVVSTLPIAHQDWLRGKEFKCKVHNKALPAPIEKTISKARGQPLEPKVYTMGPPREELSSRSVSLTCMINGFYPSDISVEWEKNGKAEDNYKTTPAVLDSDGSYFLYSKLSVPTSEWQRGDVFTCSVMHEALHNHYTQKSISRSPGK

SEQ ID NO: 10 - protein, 239 aa, oryctolagus cuniculus
MDTRAPTQLLGLLLLWLPGATFAQVLTQTASPVSAAVGGTVTINCQASQSVYDNNNLAWYQQKPGQPPKQLIYGASTLASGVSSRFKGSGSGTQFTLTISGVQCDDAATYYCLGEFSCSSADCFAFGGGTEVVVKGDPVAPTVLIFPPSADLVATGTVTIVCVANKYFPDVTVTWEVDGTTQTTGIENSKTPQNSADCTYNLSSTLTLTSTQYNSHKEYTCKVTQGTTSVVQSFNRGDC

SEQ ID NO: 11 - protein, 7 aa, oryctolagus cuniculus
LSSFAVG

SEQ ID NO: 12 - protein, 16 aa, oryctolagus cuniculus
IISSVGITRYASWAAG

SEQ ID NO: 13 - protein, 12 aa, oryctolagus cuniculus
YGYSGDVNRLDL

SEQ ID NO: 14 - protein, 11 aa, oryctolagus cuniculus
SQSVYDNNNLA

SEQ ID NO: 15 - protein, 7 aa, oryctolagus cuniculus
GASTLAS

SEQ ID NO: 16 - protein, 13 aa, oryctolagus cuniculus
LGEFSCSSADCFA

SEQ ID NO: 17 - protein, 461 aa, oryctolagus cuniculus
METGLRWLLLVAVLKGVQCQSVEESGGRLVTPGGSLTLTCTVSGFSLSDYAIIWVRQAPGKGLEYIAIIGSSGDTFYATWAKGRFTISKTSTTVDLKMTSLTAADTATYFCAPRYAGTTDYHDAFDPWGPGTLVTVSSGQPKAPSVFPLAPCCGDTPSSTVTLGCLVKGYLPEPVTVTWNSGTLTNGVRTFPSVRQSSGLYSLSSVVSVTSSSQPVTCNVAHPATNTKVDKTVAPSTCSKPTCPPPELLGGPSVFIFPPKPKDTLMISRTPEVTCVVVDVSQDDPEVQFTWYINNEQVRTARPPLREQQFNSTIRVVSTLPIAHQDWLRGKEFKCKVHNKALPAPIEKTISKARGQPLEPKVYTMGPPREELSSRSVSLTCMINGFYPSDISVEWEKNGKAEDNYKTTPAVLDSDGSYFLYSKLSVPTSEWQRGDVFTCSVMHEALHNHYTQKSISRSPGK

SEQ ID NO: 18 - protein, 238 aa, oryctolagus cuniculus
MDTRAPTQLLGLLLLWLPGARCAEVVMTQTPASMEAPMGGTVTIKCQASQNIYNYLSWYQQKPGQPPKLLVYKASTLTSGVPSRFKGSGSGTQFTLTISDLECADAATYYCQINYSIYNHYNIIFGGGTEVVVKGDPVAPTVLIFPPSADLVATGTVTIVCVANKYFPDVTVTWEVDGTTQTTGIENSKTPQNSADCTYNLSSTLTLTSTQYNSHKEYTCKVTQGTTSVVQSFNRGDC

SEQ ID NO: 19 - protein, 7 aa, oryctolagus cuniculus
LSDYAII

SEQ ID NO: 20 - protein, 16 aa, oryctolagus cuniculus
IIGSSGDTFYATWAKG

SEQ ID NO: 21 - protein, 14 aa, oryctolagus cuniculus
RYAGTTDYHDAFDP

SEQ ID NO: 22 - protein, 9 aa, oryctolagus cuniculus
SQNIYNYLS

SEQ ID NO: 23 - protein, 7 aa, oryctolagus cuniculus
KASTLTS

SEQ ID NO: 24 - protein, 13 aa, oryctolagus cuniculus
QINYSIYNHYNII

SEQ ID NO: 25 - protein, 457 aa, oryctolagus cuniculus
METGLRWLLLVAVLKGVQCQSVKESEGGLFKPTDTLTLTCTVSGFSLSSYGVTWVRQAPGNGLEWIGLIGDRGTTFYASWAKSRSTITRNTNLNTVTLKMTRLTAADTATYFCARGSGYGARIWGPGTLVTVSSWQPKAPSVFPLAPCCGDTPSSTVTLGCLVKGYLPEPVTVTWNSGTLTNGVRTFPSVRQSSGLYSLSSVVSVTSSSQPVTCNVAHPATNTKVDKTVAPSTCSKPTCPPPELLGGPSVFIFPPKPKDTLMISRTPEVTCVVVDVSQDDPEVQFTWYINNEQVRTARPPLREQQFNSTIRVVSTLPIAHQDWLRGKEFKCKVHNKALPAPIEKTISKARGQPLEPKVYTMGPPREELSSRSVSLTCMINGFYPSDISVEWEKNGKAEDNYKTTPAVLDSDGSYFLYSKLSVPTSEWQRGDVFTCSVMHEALHNHYTQKSISRSPGK

SEQ ID NO: 26 - protein, 237 aa, oryctolagus cuniculus
MDTRAPTQLLGLLLLWLPGATFAQVLTQTPSPVSAAVGGTVTINCQSSQSVYKNNYLAWYQQKPGQPPKLLIYETSKLASGVPPRFSGSGSGTQFTLTISSVQCDDAATYYCQGGYSGVDFMAFGGGTEVVVKGDPVAPTVLIFPPSADLVATGTVTIVCVANKYFPDVTVTWEVDGTTQTTGIENSKTPQNSADCTYNLSSTLTLTSTQYNSHKEYTCKVTQGTTSVVQSFNRGDC

SEQ ID NO: 27 - protein, 7 aa, oryctolagus cuniculus
LSSYGVT

SEQ ID NO: 28 - protein, 16 aa, oryctolagus cuniculus
LIGDRGTTFYASWAKS

SEQ ID NO: 29 - protein, 8 aa, oryctolagus cuniculus
GSGYGARI

SEQ ID NO: 30 - protein, 11 aa, oryctolagus cuniculus
SQSVYKNNYLA

SEQ ID NO: 31 - protein, 7 aa, oryctolagus cuniculus
ETSKLAS

SEQ ID NO: 32 - protein, 11 aa, oryctolagus cuniculus
QGGYSGVDFMA

SEQ ID NO: 33 - protein, 457 aa, oryctolagus cuniculus
METGLRWLLLVAVLKGVQCQSVKESEGGLFKPTDTLTLTCTVSGFSLTTYGVTWVRQAPGNGLEWIGLIGDRGTTYYASWVNGRSTITRNTNLNTVTLKMTRLTAADTATYFCARGSGYGARIWGPGTLVTVASWQPKAPSVFPLAPCCGDTPSSTVTLGCLVKGYLPEPVTVTWNSGTLTNGVRTFPSVRQSSGLYSLSSVVSVTSSSQPVTCNVAHPATNTKVDKTVAPSTCSKPTCPPPELLGGPSVFIFPPKPKDTLMISRTPEVTCVVVDVSQDDPEVQFTWYINNEQVRTARPPLREQQFNSTIRVVSTLPIAHQDWLRGKEFKCKVHNKALPAPIEKTISKARGQPLEPKVYTMGPPREELSSRSVSLTCMINGFYPSDISVEWEKNGKAEDNYKTTPAVLDSDGSYFLYSKLSVPTSEWQRGDVFTCSVMHEALHNHYTQKSISRSPGK

SEQ ID NO: 34 - protein, 237 aa, oryctolagus cuniculus
MDTRAPTQLLGLLLLWLPGATFAQVLTQTPSPMSAALGGTVTINCQSSQTVYNNNYLSWYQQKPGQPPKLLIYETSKLSSGVPPRFSGSGSGTQFTLTISSVQCDDAATYYCQGGYSGVDFMAFGGGTEVVVKGDPVAPTVLIFPPSADLVATGTVTIVCVANKYFPDVTVTWEVDGTTQTTGIENSKTPQNSADCTYNLSSTLTLTSTQYNSHKEYTCKVTQGTTSVVQSFNRGDC

SEQ ID NO: 35 - protein, 7 aa, oryctolagus cuniculus
LTTYGVT

SEQ ID NO: 36 - protein, 16 aa, oryctolagus cuniculus
LIGDRGTTYYASWVNG

SEQ ID NO: 37 - protein, 8 aa, oryctolagus cuniculus
GSGYGARI

SEQ ID NO: 38 - protein, 11 aa, oryctolagus cuniculus
SQTVYNNNYLS

SEQ ID NO: 39 - protein, 7 aa, oryctolagus cuniculus
ETSKLSS

SEQ ID NO: 40 - protein, 10 aa, oryctolagus cuniculus
QGGYSGVDFM

SEQ ID NO: 41 - protein, 450 aa, oryctolagus cuniculus
METGLRWLLLVAVLKGVQCQSLEESGGRLVTPGTPLTLTCTVSGFSLNNYHIYWVRQAPGKGLEYIGIIFNGGTYYARWTKGRFTISKTSTTVDLKMTSLTTEDTATYFCARGDGIWGPGTLVTVSLGQPKAPSVFPLAPCCGDTPSSTVTLGCLVKGYLPEPVTVTWNSGTLTNGVRTFPSVRQSSGLYSLSSVVSVTSSSQPVTCNVAHPATNTKVDKTVAPSTCSKPTCPPPELLGGPSVFIFPPKPKDTLMISRTPEVTCVVVDVSQDDPEVQFTWYINNEQVRTARPPLREQQFNSTIRVVSTLPIAHQDWLRGKEFKCKVHNKALPAPIEKTISKARGQPLEPKVYTMGPPREELSSRSVSLTCMINGFYPSDISVEWEKNGKAEDNYKTTPAVLDSDGSYFLYSKLSVPTSEWQRGDVFTCSVMHEALHNHYTQKSISRSPGK

SEQ ID NO: 42 - protein, 239 aa, oryctolagus cuniculus
MDTRAPTQLLGLLLLWLPGATFAQVLTQTPASVSAAVGGTVTINCQASQSVFNNNYLAWYQQKPGQPPKRLIYSASTLASGVSSRFKGSGSGTEFTLTMSGVECDDAATYYCAGSFDCNSGDCVAFGGGTEVVVKGDPVAPTVLIFPPAADQVATGTVTIVCVANKYFPDVTVTWEVDGTTQTTGIENSKTPQNSADCTYNLSSTLTLTSTQYNSHKEYTCKVTQGTTSVVQSFNRGDC

SEQ ID NO: 43 - protein, 7 aa, oryctolagus cuniculus
LNNYHIY

SEQ ID NO: 44 - protein, 15 aa, oryctolagus cuniculus
IIFNGGTYYARWTKG

SEQ ID NO: 45 - protein, 4 aa, oryctolagus cuniculus
GDGI

SEQ ID NO: 46 - protein, 11 aa, oryctolagus cuniculus
SQSVFNNNYLA

SEQ ID NO: 47 - protein, 7 aa, oryctolagus cuniculus
SASTLAS

SEQ ID NO: 48 - protein, 13 aa, oryctolagus cuniculus
AGSFDCNSGDCVA

SEQ ID NO: 49 - DNA, 1029 bp, homo sapiens
atggcgcaggtgctgatcgtgggcgccgggatgacaggaagcttgtgcgctgcgctgctgaggaggcagacgtccggtcccttgtaccttgctgtgtgggacaaggctgaggactcagggggaagaatgactacagcctgcagtcctcataatcctcagtgcacagctgacttgggtgctcagtacatcacctgcactcctcattatgccaaaaaacaccaacgtttttatgatgaactgttagcctatggcgttttgaggcctctaagctcgcctattgaaggaatggtgatgaaagaaggagactgtaactttgtggcacctcaaggaatttcttcaattattaagcattacttgaaagaatcaggtgcagaagtctacttcagacatcgtgtgacacagatcaacctaagagatgacaaatgggaagtatccaaacaaacaggctcccctgagcagtttgatcttattgttctcacaatgccagttcctgagattctgcagcttcaaggtgacatcaccaccttaattagtgaatgccaaaggcagcaactggaggctgtgagctactcctctcgatatgctctgggcctcttttatgaagctggtacgaagattgatgtcccttgggctgggcagtacatcaccagtaatccctgcatacgcttcgtctccattgataataagaagcgcaatatagagtcatcagaaattgggccttccctcgtgattcacaccactgtcccatttggagttacatacttggaacacagcattgaggatgtgcaagagttagtcttccagcagctggaaaacattttgccgggtttgcctcagccaattgctaccaaatgccaaaaatggagacattcacaggttacaaatgctgctgccaactgtcctggccaaatgactctgcatcacaaacctttccttgcatgtggaggggatggatttactcagtccaactttgatggctgcatcacttctgccctatgtgttctggaagctttaaagaattatatttaa

SEQ ID NO: 50 - protein, 315 aa, homo sapiens
MAQVLIVGAGMTGSLCAALLRRQTSGPLYLAVWDKAEDSGGRMTTACSPHNPQCTADLGAQYITCTPHYAKKHQRFYDELLAYGVLRPLSSPIEGMVMKEGDCNFVAPQGISSIIKHYLKESGAEVYFRHRVTQINLRDDKWEVSKQTGSPEQFDLIVLTMPVPEILQLQGDITTLISECQRQQLEAVSYSSRYALGLFYEAGTKIDVPWAGQYITSNPCIRFVSIDNKKRNIESSEIGPSLVIHTTVPFGVTYLEHSIEDVQELVFQQLENILPGLPQPIATKCQKWRHSQVPSAGVILGCAKSPWMMAIGFPI

SEQ ID NO: 51 - DNA, 945 bp, homo sapiens
atggcgcaggtgctgatcgtgggcgccgggatgacaggaagcttgtgcgctgcgctgctgaggaggcagacgtccggtcccttgtaccttgctgtgtgggacaaggctgaggactcagggggaagaatgactacagcctgcagtcctcataatcctcagtgcacagctgacttgggtgctcagtacatcacctgcactcctcattatgccaaaaaacaccaacgtttttatgatgaactgttagcctatggcgttttgaggcctctaagctcgcctattgaaggaatggtgatgaaagaaggagactgtaactttgtggcacctcaaggaatttcttcaattattaagcattacttgaaagaatcaggtgcagaagtctacttcagacatcgtgtgacacagatcaacctaagagatgacaaatgggaagtatccaaacaaacaggctcccctgagcagtttgatcttattgttctcacaatgccagttcctgagattctgcagcttcaaggtgacatcaccaccttaattagtgaatgccaaaggcagcaactggaggctgtgagctactcctctcgatatgctctgggcctcttttatgaagctggtacgaagattgatgtcccttgggctgggcagtacatcaccagtaatccctgcatacgcttcgtctccattgataataagaagcgcaatatagagtcatcagaaattgggccttccctcgtgattcacaccactgtcccatttggagttacatacttggaacacagcattgaggatgtgcaagagttagtcttccagcagctggaaaacattttgccgggtttgcctcagccaattgctaccaaatgccaaaaatggagacattcacaggtaccaagtgctggtgtgattctaggatgtgcgaagagcccctggatgatggcgattggatttcccatc

SEQ ID NO: 52 - DNA, 1380 bp, oryctolagus cuniculus
atggagactgggctgcgctggcttctcctggtcgctgtgctcaaaggtgtccagtgtcagtcggtggaggagtccgggggtcgcctggtcacgcctgggacacccctgacactcacctgcacagtctctggattctccctcagtagttttgcagtgggctgggtccgccaggctccagggaaggggctggaatacatcggaatcattagtagtgttggtattacacgctacgcgagctgggcggccggccgattcaccatctccaaaacctcgaccacggtggatctgaaaatcaccagtccgacaaccgaggacacggccacctatttttgtgccagatatggttatagtggtgatgttaatcggttggatctctggggccagggcaccctggtcaccgtctcctcagggcaacctaaggctccatcagtcttcccactggccccctgctgcggggacacacccagctccacggtgaccctgggctgcctggtcaaagggtacctcccggagccagtgaccgtgacctggaactcgggcaccctcaccaatggggtacgcaccttcccgtccgtccggcagtcctcaggcctctactcgctgagcagcgtggtgagcgtgacctcaagcagccagcccgtcacctgcaacgtggcccacccagccaccaacaccaaagtggacaagaccgttgcgccctcgacatgcagcaagcccacgtgcccaccccctgaactcctggggggaccgtctgtcttcatcttccccccaaaacccaaggacaccctcatgatctcacgcacccccgaggtcacatgcgtggtggtggacgtgagccaggatgaccccgaggtgcagttcacatggtacataaacaacgagcaggtgcgcaccgcccggccgccgctacgggagcagcagttcaacagcacgatccgcgtggtcagcaccctccccatcgcgcaccaggactggctgaggggcaaggagttcaagtgcaaagtccacaacaaggcactcccggcccccatcgagaaaaccatctccaaagccagagggcagcccctggagccgaaggtctacaccatgggccctccccgggaggagctgagcagcaggtcggtcagcctgacctgcatgatcaacggcttctacccttccgacatctcggtggagtgggagaagaacgggaaggcagaggacaactacaagaccacgccggccgtgctggacagcgacggctcctacttcctctacagcaagctctcagtgcccacgagtgagtggcagcggggcgacgtcttcacctgctccgtgatgcacgaggccttgcacaaccactacacgcagaagtccatctcccgctctccgggtaaatga

SEQ ID NO: 53 - DNA, 720 bp, oryctolagus cuniculus
atggacacgagggcccccactcagctgctggggctcctgctgctctggctcccaggtgccacatttgcccaagtgctgacccagactgcatcgcccgtgtctgcagctgtgggaggcacagtcaccatcaattgccaggccagtcagagtgtttatgataacaacaacttagcctggtatcagcagaaaccagggcagcctcccaagcaactgatctatggtgcatccactctggcatctggggtctcatcgcggttcaaaggcagtggatctgggacacagttcactctcaccatcagcggcgtgcagtgtgacgatgctgccacttactactgtctaggcgaatttagttgtagtagtgctgattgttttgctttcggcggagggaccgaggtggtcgtcaaaggtgatccagttgcacctactgtcctcatcttcccaccatctgctgatcttgtggcaactggaacagtcaccatcgtgtgtgtggcgaataaatactttcccgatgtcaccgtcacctgggaggtggatggcaccacccaaacaactggcatcgagaacagtaaaacaccgcagaattctgcagattgtacctacaacctcagcagcactctgacactgaccagcacacagtacaacagccacaaagagtacacctgcaaggtgacccagggcacgacctcagtcgtccagagcttcaataggggtgactgttag

SEQ ID NO: 54 - DNA, 21 bp, oryctolagus cuniculus
ctcagtagttttgcagtgggc

SEQ ID NO: 55 - DNA, 48 bp, oryctolagus cuniculus
atcattagtagtgttggtattacacgctacgcgagctgggcggccggc

SEQ ID NO: 56 - DNA, 36 bp, oryctolagus cuniculus
tatggttatagtggtgatgttaatcggttggatctc

SEQ ID NO: 57 - DNA, 33 bp, oryctolagus cuniculus
agtcagagtgtttatgataacaacaacttagcc

SEQ ID NO: 58 - DNA, 21 bp, oryctolagus cuniculus
ggtgcatccactctggcatct

SEQ ID NO: 59 - DNA, 39 bp, oryctolagus cuniculus
ctaggcgaatttagttgtagtagtgctgattgttttgct

SEQ ID NO: 60 - DNA, 1386 bp, oryctolagus cuniculus
atggagactgggctgcgctggcttctcctggtcgctgtgctcaaaggtgtccagtgtcagtcggtggaggagtccgggggtcgcctggtcacgcctggaggatccctgacactcacctgcacagtctctggattctccctcagtgactatgcaataatctgggtccgccaggctccagggaaggggctggaatacatcgcaattattggtagtagtggtgacacattctacgcgacctgggcgaaaggccgattcaccatctccaaaacctcgaccacggtggatctgaaaatgaccagtctgacagccgcggacacggccacctatttctgtgccccacgttatgctggtactactgattatcatgatgcttttgatccctggggcccaggcactttggtcaccgtctcctcagggcaacctaaggctccatcagtcttcccactggccccctgctgcggggacacacccagctccacggtgaccctgggctgcctggtcaaagggtacctcccggagccagtgaccgtgacctggaactcgggcaccctcaccaatggggtacgcaccttcccgtccgtccggcagtcctcaggcctctactcgctgagcagcgtggtgagcgtgacctcaagcagccagcccgtcacctgcaacgtggcccacccagccaccaacaccaaagtggacaagaccgttgcgccctcgacatgcagcaagcccacgtgcccaccccctgaactcctggggggaccgtctgtcttcatcttccccccaaaacccaaggacaccctcatgatctcacgcacccccgaggtcacatgcgtggtggtggacgtgagccaggatgaccccgaggtgcagttcacatggtacataaacaacgagcaggtgcgcaccgcccggccgccgctacgggagcagcagttcaacagcacgatccgcgtggtcagcaccctccccatcgcgcaccaggactggctgaggggcaaggagttcaagtgcaaagtccacaacaaggcactcccggcccccatcgagaaaaccatctccaaagccagagggcagcccctggagccgaaggtctacaccatgggccctccccgggaggagctgagcagcaggtcggtcagcctgacctgcatgatcaacggcttctacccttccgacatctcggtggagtgggagaagaacgggaaggcagaggacaactacaagaccacgccggccgtgctggacagcgacggctcctacttcctctacagcaagctctcagtgcccacgagtgagtggcagcggggcgacgtcttcacctgctccgtgatgcacgaggccttgcacaaccactacacgcagaagtccatctcccgctctccgggtaaatga

SEQ ID NO: 61 - DNA, 717 bp, oryctolagus cuniculus
atggacacgagggcccccactcagctgctggggctcctgctgctctggctcccaggtgccagatgtgccgaagtagtgatgacccagactccagcctccatggaggcacctatgggaggcacagtcaccatcaagtgccaggccagtcagaacatttacaactacttatcctggtatcagcagaaaccagggcagcctcccaagctcctagtctacaaggcctccactctgacttctggggtcccgtcgcgcttcaaaggcagtggatctgggacacagttcactctcaccatcagcgacctggagtgtgccgatgctgccacttactactgtcaaatcaattactctatttataatcattataatattatttttggcggagggaccgaggtggtcgtcaagggtgatccagttgcacctactgtcctcatcttcccaccatctgctgatcttgtggcaactggaacagtcaccatcgtgtgtgtggcgaataaatactttcccgatgtcaccgtcacctgggaggtggatggcaccacccaaacaactggcatcgagaacagtaaaacaccgcagaattctgcagattgtacctacaacctcagcagcactctgacactgaccagcacacagtacaacagccacaaagagtacacctgcaaggtgacccagggcacgacctcagtcgtccagagcttcaataggggtgactgttag

SEQ ID NO: 62 - DNA, 21 bp, oryctolagus cuniculus
ctcagtgactatgcaataatc

SEQ ID NO: 63 - DNA, 48 bp, oryctolagus cuniculus
attattggtagtagtggtgacacattctacgcgacctgggcgaaaggc

SEQ ID NO: 64 - DNA, 42 bp, oryctolagus cuniculus
cgttatgctggtactactgattatcatgatgcttttgatccc

SEQ ID NO: 65 - DNA, 27 bp, oryctolagus cuniculus
agtcagaacatttacaactacttatcc

SEQ ID NO: 66 - DNA, 21 bp, oryctolagus cuniculus
aaggcctccactctgacttct

SEQ ID NO: 67 - DNA, 39 bp, oryctolagus cuniculus
caaatcaattactctatttataatcattataatattatt

SEQ ID NO: 68 - DNA, 1374 bp, oryctolagus cuniculus
atggagactgggctgcgctggcttctcctggtcgctgtgctcaaaggtgtccagtgtcagtcggtgaaggagtccgagggaggtctcttcaagccaacggataccctgacactcacctgcacagtctctggattctccctcagtagctatggagtgacctgggtccgccaggctccagggaacgggctggagtggatcggattgattggtgatcgtggtactacgttctacgcgagctgggcgaaaagccgatccaccatcaccagaaacaccaacctgaacacggtgactctgaaaatgaccaggctgacagccgcggacacggccacctatttctgtgcgagggggagtgggtatggtgctcgcatctggggcccaggcaccctggtcaccgtctcctcatggcaacctaaggctccatcagtcttcccactggccccctgctgcggggacacacccagctccacggtgaccctgggctgcctggtcaaagggtacctcccggagccagtgaccgtgacctggaactcgggcaccctcaccaatggggtacgcaccttcccgtccgtccggcagtcctcaggcctctactcgctgagcagcgtggtgagcgtgacctcaagcagccagcccgtcacctgcaacgtggcccacccagccaccaacaccaaagtggacaagaccgttgcgccctcgacatgcagcaagcccacgtgcccaccccctgaactcctggggggaccgtctgtcttcatcttccccccaaaacccaaggacaccctcatgatctcacgcacccccgaggtcacatgcgtggtggtggacgtgagccaggatgaccccgaggtgcagttcacatggtacataaacaacgagcaggtgcgcaccgcccggccgccgctacgggagcagcagttcaacagcacgatccgcgtggtcagcaccctccccatcgcgcaccaggactggctgaggggcaaggagttcaagtgcaaagtccacaacaaggcactcccggcccccatcgagaaaaccatctccaaagccagagggcagcccctggagccgaaggtctacaccatgggccctccccgggaggagctgagcagcaggtcggtcagcctgacctgcatgatcaacggcttctacccttccgacatctcggtggagtgggagaagaacgggaaggcagaggacaactacaagaccacgccggccgtgctggacagcgacggctcctacttcctctacagcaagctctcagtgcccacgagtgagtggcagcggggcgacgtcttcacctgctccgtgatgcacgaggccttgcacaaccactacacgcagaagtccatctcccgctctccgggtaaatga

SEQ ID NO: 69 - DNA, 714 bp, oryctolagus cuniculus
atggacacgagggcccccactcagctcctggggctcctgctgctctggctcccaggtgccacatttgcccaagtgctgacccagactccatcgcctgtgtctgcagctgtgggaggcacagtcaccatcaattgccagtccagtcagagtgtttataagaacaactacttagcctggtatcagcagaaaccagggcagcctcccaagctccttatctacgaaacatccaaactggcatctggggtcccaccgcggttcagcggcagtgggtctgggacacagttcactctcaccatcagcagcgtgcagtgtgacgatgctgccacttactactgtcaaggcggttatagtggtgttgattttatggctttcggcggagggaccgaggtggtcgtcaaaggtgatccagttgcacctactgtcctcatcttcccaccatctgctgatcttgtggcaactggaacagtcaccatcgtgtgtgtggcgaataaatactttcccgatgtcaccgtcacctgggaggtggatggcaccacccaaacaactggcatcgagaacagtaaaacaccgcagaattctgcagattgtacctacaacctcagcagcactctgacactgaccagcacacagtacaacagccacaaagagtacacctgcaaggtgacccagggcacgacctcagtcgtccagagcttcaataggggtgactgttag

SEQ ID NO: 70 - DNA, 21 bp, oryctolagus cuniculus
ctcagtagctatggagtgacc

SEQ ID NO: 71 - DNA, 48 bp, oryctolagus cuniculus
ttgattggtgatcgtggtactacgttctacgcgagctgggcgaaaagc

SEQ ID NO: 72 - DNA, 24 bp, oryctolagus cuniculus
gggagtgggtatggtgctcgcatc

SEQ ID NO: 73 - DNA, 33 bp, oryctolagus cuniculus
agtcagagtgtttataagaacaactacttagcc

SEQ ID NO: 74 - DNA, 21 bp, oryctolagus cuniculus
gaaacatccaaactggcatct

SEQ ID NO: 75 - DNA, 33 bp, oryctolagus cuniculus
caaggcggttatagtggtgttgattttatggct

SEQ ID NO: 76 - DNA, 1374 bp, oryctolagus cuniculus
atggagactgggctgcgctggcttctcctggtcgctgtgctcaaaggtgtccagtgtcagtcggtgaaggagtccgagggaggtctcttcaagccaacggataccctgacactcacctgcacagtctctggattctccctcactacctatggagtgacctgggtccgccaggctccagggaatgggctggagtggatcggattgattggtgatcgcggtaccacttactacgcgagctgggtgaatggccgatccaccatcaccagaaacaccaacctgaacacggtgactctgaaaatgaccaggctgacagccgcggacacggccacctatttctgtgcgagggggagtggatatggtgctcgcatctggggcccaggcaccctggtcaccgtcgcctcatggcaacctaaggctccatcagtcttcccactggccccctgctgcggggacacacccagctccacggtgaccctgggctgcctggtcaaagggtacctcccggagccagtgaccgtgacctggaactcgggcaccctcaccaatggggtacgcaccttcccgtccgtccggcagtcctcaggcctctactcgctgagcagcgtggtgagcgtgacctcaagcagccagcccgtcacctgcaacgtggcccacccagccaccaacaccaaagtggacaagaccgttgcgccctcgacatgcagcaagcccacgtgcccaccccctgaactcctggggggaccgtctgtcttcatcttccccccaaaacccaaggacaccctcatgatctcacgcacccccgaggtcacatgcgtggtggtggacgtgagccaggatgaccccgaggtgcagttcacatggtacataaacaacgagcaggtgcgcaccgcccggccgccgctacgggagcagcagttcaacagcacgatccgcgtggtcagcaccctccccatcgcgcaccaggactggctgaggggcaaggagttcaagtgcaaagtccacaacaaggcactcccggcccccatcgagaaaaccatctccaaagccagagggcagcccctggagccgaaggtctacaccatgggccctccccgggaggagctgagcagcaggtcggtcagcctgacctgcatgatcaacggcttctacccttccgacatctcggtggagtgggagaagaacgggaaggcagaggacaactacaagaccacgccggccgtgctggacagcgacggctcctacttcctctacagcaagctctcagtgcccacgagtgagtggcagcggggcgacgtcttcacctgctccgtgatgcacgaggccttgcacaaccactacacgcagaagtccatctcccgctctccgggtaaatga

SEQ ID NO: 77 - DNA, 714 bp, oryctolagus cuniculus
atggacacgagggcccccactcagctcctggggctcctgctgctctggctcccaggtgccacatttgcccaagtgctgacccagactccatcccccatgtctgcagctctgggaggcacagtcaccatcaattgccagtccagtcagactgtttataacaataactacttatcctggtatcagcagaaaccagggcagcctcccaagctccttatctacgaaacatccaaactgtcatctggggtcccaccgcggttcagcggcagtgggtctgggacacagttcactctcaccatcagcagcgtgcagtgtgacgatgctgccacttactactgtcaaggcggttatagtggtgttgattttatggctttcggcggagggaccgaggtggtcgtcaaaggtgatccagttgcacctactgtcctcatcttcccaccatctgctgatcttgtggcaactggaacagtcaccatcgtgtgtgtggcgaataaatactttcccgatgtcaccgtcacctgggaggtggatggcaccacccaaacaactggcatcgagaacagtaaaacaccgcagaattctgcagattgtacctacaacctcagcagcactctgacactgaccagcacacagtacaacagccacaaagagtacacctgcaaggtgacccagggcacgacctcagtcgtccagagcttcaataggggtgactgttag

SEQ ID NO: 78 - DNA, 21 bp, oryctolagus cuniculus
ctcactacctatggagtgacc

SEQ ID NO: 79 - DNA, 48 bp, oryctolagus cuniculus
ttgattggtgatcgcggtaccacttactacgcgagctgggtgaatggc

SEQ ID NO: 80 - DNA, 24 bp, oryctolagus cuniculus
gggagtggatatggtgctcgcatc

SEQ ID NO: 81 - DNA, 33 bp, oryctolagus cuniculus
agtcagactgtttataacaataactacttatcc

SEQ ID NO: 82 - DNA, 21 bp, oryctolagus cuniculus
gaaacatccaaactgtcatct

SEQ ID NO: 83 - DNA, 30 bp, oryctolagus cuniculus
ggcggttatagtggtgttgattttatggct

SEQ ID NO: 84 - DNA, 1353 bp, oryctolagus cuniculus
atggagactgggctgcgctggcttctcctggtcgctgtgctcaaaggtgtccagtgtcagtcgctggaggagtccgggggtcgcctggtcacgcctgggacacccctgacactcacctgcacagtctctggattctccctcaataactaccacatatactgggtccgccaggctccaggaaaggggctggaatacatcggaatcattttcaatggtggcacatattacgcgagatggacaaaaggccgattcaccatctccaaaacctcgaccacggtggatctgaaaatgaccagtctgacaaccgaggacacggccacctatttctgtgccagaggggacggcatctggggcccaggcaccctggtcaccgtctccttagggcaacctaaggctccatcagtcttcccactggccccctgctgcggggacacacccagctccacggtgaccctgggctgcctggtcaaagggtacctcccggagccagtgaccgtgacctggaactcgggcaccctcaccaatggggtacgcaccttcccgtccgtccggcagtcctcaggcctctactcgctgagcagcgtggtgagcgtgacctcaagcagccagcccgtcacctgcaacgtggcccacccagccaccaacaccaaagtggacaagaccgttgcgccctcgacatgcagcaagcccacgtgcccaccccctgaactcctggggggaccgtctgtcttcatcttccccccaaaacccaaggacaccctcatgatctcacgcacccccgaggtcacatgcgtggtggtggacgtgagccaggatgaccccgaggtgcagttcacatggtacataaacaacgagcaggtgcgcaccgcccggccgccgctacgggagcagcagttcaacagcacgatccgcgtggtcagcaccctccccatcgcgcaccaggactggctgaggggcaaggagttcaagtgcaaagtccacaacaaggcactcccggcccccatcgagaaaaccatctccaaagccagagggcagcccctggagccgaaggtctacaccatgggccctccccgggaggagctgagcagcaggtcggtcagcctgacctgcatgatcaacggcttctacccttccgacatctcggtggagtgggagaagaacgggaaggcagaggacaactacaagaccacgccggccgtgctggacagcgacggctcctacttcctctacagcaagctctcagtgcccacgagtgagtggcagcggggcgacgtcttcacctgctccgtgatgcacgaggccttgcacaaccactacacgcagaagtccatctcccgctctccgggtaaatga

SEQ ID NO: 85 - DNA, 720 bp, oryctolagus cuniculus
atggacacgagggcccccactcagctgctggggctcctgctgctctggctcccaggtgccacatttgcccaagtgctgacccagactccagcctccgtgtctgcagctgtgggaggcacagtcaccatcaattgccaggccagtcagagtgtttttaataacaactatttagcctggtatcagcagaaaccagggcagcctcccaagcgcctgatctattctgcatccactctggcgtctggggtctcatcgcggttcaaaggcagtggatctgggacagaattcactctgaccatgagtggcgtggagtgtgacgatgctgccacttactactgtgcaggcagttttgattgtaatagtggtgattgtgttgctttcggcggagggaccgaggtggtggtcaagggtgatccagttgcacctactgtcctcatcttcccaccagctgctgatcaggtggcaactggaacagtcaccatcgtgtgtgtggcgaataaatactttcccgatgtcaccgtcacctgggaggtggatggcaccacccaaacaactggcatcgagaacagtaaaacaccgcagaattctgcagattgtacctacaacctcagcagcactctgacactgaccagcacacagtacaacagccacaaagagtacacctgcaaggtgacccagggcacgacctcagtcgtccagagcttcaataggggtgactgttag

SEQ ID NO: 86 - DNA, 21 bp, oryctolagus cuniculus
ctcaataactaccacatatac

SEQ ID NO: 87 - DNA, 45 bp, oryctolagus cuniculus
atcattttcaatggtggcacatattacgcgagatggacaaaaggc

SEQ ID NO: 88 - DNA, 12 bp, oryctolagus cuniculus
ggggacggcatc

SEQ ID NO: 89 - DNA, 33 bp, oryctolagus cuniculus
agtcagagtgtttttaataacaactatttagcc

SEQ ID NO: 90 - DNA, 21 bp, oryctolagus cuniculus
tctgcatccactctggcgtct

SEQ ID NO: 91 - DNA, 39 bp, oryctolagus cuniculus
gcaggcagttttgattgtaatagtggtgattgtgttgct

SEQ ID NO: 92 - protein, 342 aa, homo sapiens
MAQVLIVGAGMTGSLCAALLRRQTSGPLYLAVWDKADDSGGRMTTACSPHNPQCTADLGAQYITCTPHYAKKHQRFYDELLAYGVLRPLSSPIEGMVMKEGDCNFVAPQGISSIIKHYLKESGAEVYFRHRVTQINLRDDKWEVSKQTGSPEQFDLIVLTMPVPEILQLQGDITTLISECQRQQLEAVSYSSRYALGLFYEAGTKIDVPWAGQYITSNPCIRFVSIDNKKRNIESSEIGPSLVIHTTVPFGVTYLEHSIEDVQELVFQQLENILPGLPQPIATKCQKWRHSQVTNAAANCPGQMTLHHKPFLACGGDGFTQSNFDGCITSALCVLEALKNYI

SEQ ID NO: 93 - DNA, 1029 bp, homo sapiens
atggcgcaggtgctgatcgtgggcgccgggatgacaggaagcttgtgcgctgcgctgctgacgaggcagacgtccggtcccttgtaccttgctgtgtgggacaaggctgaggactcagggggaagaatgactacagcctgcagtcctcataatcctcagtgcacagctgacttgggtgctcagtacatcacctgcactcctcattatgccaaaaaacaccaacgtttttatgatgaactgttagcctatggcgttttgaggcctctaagctcgcctattgaaggaatggtgatgaaagaaggagactgtaactttgtggcacctcaaggaatttcttcaattattaagcattacttgaaagaatcaggtgcagaagtctacttcagacatcgtgtgacacagatcaacctaagagatgacaaatgggaagtatccaaacaaacaggctcccctgagcagtttgatcttattgttctcacaatgccagttcctgagattctgcagcttcaaggtgacatcaccaccttaattagtgaatgccaaaggcagcaactggaggctgtgagctactcctctcgatatgctctgggcctcttttatgaagctggtacgaagattgatgtcccttgggctgggcagtacatcaccagtaatccctgcatacgcttcgtctccattgataataagaagcgcaatatagagtcatcagaaattgggccttccctcgtgattcacaccactgtcccatttggagttacatacttggaacacagcattgaggatgtgcaagagttagtcttccagcagctggaaaacattttgccgggtttgcctcagccaattgctaccaaatgccaaaaatggagacattcacaggttacaaatgctgctgccaactgtcctggccaaatgactctgcatcacaaacctttccttgcatgtggaggggatggatttactcagtccaactttgatggctgcatcacttctgccctatgtgttctggaagctttaaagaattatatttaa

SEQ ID NO: 94 - protein, 315 aa, homo sapiens
MAQVLIVGAGMTGSLCAALLRRQTSGPLYLAVWDKADDSGGRMTTACSPHNPQCTADLGAQYITCTPHYAKKHQRFYDELLAYGVLRPLSSPIEGMVMKEGDCNFVAPQGISSIIKHYLKESGAEVYFRHRVTQINLRDDKWEVSKQTGSPEQFDLIVLTMPVPEILQLQGDITTLISECQRQQLEAVSYSSRYALGLFYEAGTKIDVPWAGQYITSNPCIRFVSIDNKKRNIESSEIGPSLVIHTTVPFGVTYLEHSIEDVQELVFQQLENILPGLPQPIATKCQKWRHSQVPSAGVILGCAKSPWMMAIGFPI

SEQ ID NO: 95 - DNA, 945 bp, homo sapiens
atggcgcaggtgctgatcgtgggcgccgggatgacaggaagcttgtgcgctgcgctgctgacgaggcagacgtccggtcccttgtaccttgctgtgtgggacaaggctgaggactcagggggaagaatgactacagcctgcagtcctcataatcctcagtgcacagctgacttgggtgctcagtacatcacctgcactcctcattatgccaaaaaacaccaacgtttttatgatgaactgttagcctatggcgttttgaggcctctaagctcgcctattgaaggaatggtgatgaaagaaggagactgtaactttgtggcacctcaaggaatttcttcaattattaagcattacttgaaagaatcaggtgcagaagtctacttcagacatcgtgtgacacagatcaacctaagagatgacaaatgggaagtatccaaacaaacaggctcccctgagcagtttgatcttattgttctcacaatgccagttcctgagattctgcagcttcaaggtgacatcaccaccttaattagtgaatgccaaaggcagcaactggaggctgtgagctactcctctcgatatgctctgggcctcttttatgaagctggtacgaagattgatgtcccttgggctgggcagtacatcaccagtaatccctgcatacgcttcgtctccattgataataagaagcgcaatatagagtcatcagaaattgggccttccctcgtgattcacaccactgtcccatttggagttacatacttggaacacagcattgaggatgtgcaagagttagtcttccagcagctggaaaacattttgccgggtttgcctcagccaattgctaccaaatgccaaaaatggagacattcacaggtaccaagtgctggtgtgattctaggatgtgcgaagagcccctggatgatggcgattggatttcccatc